European Patent Specification EP 3 220 937 B1, published September 4, 2024. Title: PNEUMOLYSIN MUTANTS AND METHODS OF USE THEREOF. Applicant: The Board of Regents of the University of Oklahoma. The sequence listing filed with the application follows.

SEQUENCE LISTING (40 sequences)

SEQ ID NO: 1 - protein, 471 aa, Streptococcus pneumoniae
MANKAVNDFILAMNYDKKKLLTHQGESIENRFIKEGNQLPDEFVVIERKKRSLSTNTSDISVTATNDSRLYPGALLVVDETLLENNPTLLAVDRAPMTYSIDLPGLASSDSFLQVEDPSNSSVRGAVNDLLAKWHQDYGQVNNVPARMQYEKITAHSMEQLKVKFGSDFEKTGNSLDIDFNSVHSGEKQIQIVNFKQIYYTVSVDAVKNPGDVFQDTVTVEDLKQRGISAERPLVYISSVAYGRQVYLKLETTSKSDEVEAAFEALIKGVKVAPQTEWKQILDNTEVKAVILGGDPSSGARVVTGKVDMVEDLIQEGSRFTADHPGLPISYTTSFLRDNVVATFQNSTDYVETKVTAYRNGDLLLDHSGAYVAQYYITWDELSYDHQGKEVLTPKAWDRNGQDLTAHFTTSIPLKGNVRNLSVKIRECTGLAWEWWRTVYEKTDLPLVRKRTISIWGTTLYPQVEDKVEND

SEQ ID NO: 2 - protein, 509 aa, Bacillus cereus
MNIKKNTKRRKFLACLLVSLCTINYSSISFAETQASNATDVTKNASGIDTGIANLKYNNQEVLAVNGDKVESFVPKESINSNGKFVVVEREKKSLTTSPVDISIIDSVVNRTYPGAVQLANKAFADNQPSLLVAKRKPLNISIDLPGMRKENTITVQNPTYGNVAGAVDDLVSTWNEKYSTTHTLPARMQYTESMVYSKSQIASALNVNAKYLDNSLNIDFNAVANGEKKVMVAAYKQIFYTVSAELPNNPSDLFDNSVTFDELTRKGVSNSAPPVMVSNVAYGRTIYVKLETTSKSKDVQAAFKALLKNNSVETSGQYKDIFEESTFTAVVLGGDAKEHNKVVTKDFNEIRNIIKDNAELSLKNPAYPISYTSTFLKDNSTAAVHNNTDYIETTTTEYSSAKMTLDHYGAYVAQFDVSWDEFTFDQKGNEVLTHKTWDGSGKDKTAHYSTVIPLPPNSKNIKIVARECTGLAWEWWRTIINEQNVPLTNEIKVSIGGTTLYPTASISH

SEQ ID NO: 3 - protein, 512 aa, Bacillus anthracis
MIFLNIKKNTKRRKFLACLLVSLCTIHYSSISFAETQAGNATGAIKNASDINTGIANLKYDSRDILAVNGDKVESFIPKESINSNGKFVVVEREKKSLTTSPVDILIIDSVVNRTYPGAVQLANKAFADNQPSLLVAKRKPLNISIDLPGMRKENTITVQNPTYGNVAGAVDDLVSTWNEKYSTTHTLPARMQYTESMVYSKSQIASALNVNAKYLDNSLNIDFNAVANGEKKVMVAAYKQIFYTVSAELPNNPSDLFDNSVTFDELTRKGVSNSAPPVMVSNVAYGRTVYVKLETTSKSKDVQAAFKALLKNNSVETSGQYKDIFEESTFTAVVLGGDAKEHNKVVTKDFNEIRNIIKDNAELSFKNPAYPISYTSTFLKDNATAAVHNNTDYIETTTTEYSSAKMTLDHYGAYVAQFDVSWDEFTFDQNGKEVLTHKTWEGSGKDKTAHYSTVIPLPPNSKNIKIVARECTGLAWEWWRTIINEQNVPLTNEIKVSIGGTTLYPTATISH

SEQ ID NO: 4 - protein, 509 aa, Bacillus thuringiensis
MNIKKNTKRRKFLACLLVSLCTINYSSISFAETQASNATDVTKNASGIDTGIANLKYNIQEVLAVNGDKVESFVPKESINSNGKFVVVEREKKSLTTSPVDISIIDSVVNRTYPGAVQLANKAFADNQPSLLVAKRKPLNISIDLPGMRKENTITVQNPTYGNVAGAVDDLVSTWNEKYSTTHTLPARMQYTESMVYSKSQIASALNVNAKYLDNSLNIGFNAVANGEKKVMVAAYKQIFYTVSAELPNNPSDLFDNSVTFDELTRKGVNNSAPPVMVSNVAYGRTIYVKLETTSKSKDVQAAFKALLKNNSVETSGQYKDIFEESTFTAVVLGGDAKEHNKVVTKDFNEIRNIIKDNAELSLKNPAYPISYTSTFLKDNATAAVHNNTDYIETTTTEYSSAKMTLDHYGAYVAQFDVSWDEFTFDQKGNEVLTHKTWDGSGKDKTAHYSTVIPLPPNSKNIKIVARECTGLAWEWWRTIINEQNVPLTNEIKVSIGGTTLYPTASISH

SEQ ID NO: 5 - protein, 500 aa, Clostridium perfringens
MIRFKKTKLIASIAMALCLFSQPVISFSKDITDKNQSIDSGISSLSYNRNEVLASNGDKIESFVPKEGKKAGNKFIVVERQKRSLTTSPVDISIIDSVNDRTYPGALQLADKAFVENRPTILMVKRKPININIDLPGLKGENSIKVDDPTYGKVSGAIDELVSKWNEKYSSTHTLPARTQYSESMVYSKSQISSALNVNAKVLENSLGVDFNAVANNEKKVMILAYKQIFYTVSADLPKNPSDLFDDSVTFNDLKQKGVSNEAPPLMVSNVAYGRTIYVKLETTSSSKDVQAAFKALIKNTDIKNSQQYKDIYENSSFTAVVLGGDAQEHNKVVTKDFDEIRKVIKDNATFSTKNPAYPISYTSVFLKDNSVAAVHNKTDYIETTSTEYSKGKINLDHSGAYVAQFEVAWDEVSYDKEGNEVLTHKTWDGNYQDKTAHYSTVIPLEANARNIRIKARECTGLAWEWWRDVISEYDVPLTNNINVSIWGTTLYPGSSITYN

SEQ ID NO: 6 - protein, 501 aa, Bacillus alvei
MKKKSNHLKGRKVLVSLLVSLQVFAFASISSAAPTEPNDIDMGIAGLNYNRNEVLAIQGDQISSFVPKEGIQSNGKFIVVERDKKSLTTSPVDISIVDSITNRTYPGAIQLANKDFADNQPSLVMAARKPLDISIDLPGLKNENTISVQNPNYGTVSSAIDQLVSTWGEKYSSTHTLPARLQYAESMVYSQNQISSALNVNAKVLNGTLGIDFNAVANGEKKVMVAAYKQIFYTVSAGLPNNPSDLFDDSVTFAELARKGVSNEAPPLMVSNVAYGRTIYVKLETTSKSNDVQTAFKLLLNNPSIQASGQYKDIYENSSFTAVVLGGDAQTHNQVVTKDFNVIQSVIKDNAQFSSKNPAYPISYTSVFLKDNSIAAVHNNTEYIETKTTEYSKGKIKLDHSGAYVAQFEVYWDEFSYDADGQEIVTRKSWDGNWRDRSAHFSTEIPLPPNAKNIRIFARECTGLAWEWWRTVVDEYNVPLASDINVSIWGTTLYPKSSITH

SEQ ID NO: 7 - protein, 574 aa, Streptococcus canis
MKDMSNKKIFKKYSRVAGLLTAALIVGNLVTANADSNKQNTANTETTTTNEQPKPESSELTTEKAGQKMDDMLNSNDMIKLAPKEMPLESAEKEEKKSEDNKKSEEDHTEEINDKIYSLNYNELEVLAKNGETIENFVPKEGVKKADKFIVIERKKKNINTTPVDISIIDSVTDRTYPAALQLANKGFTENKPDAVVTKRNPQKIHIDLPGMGDKATVEVNDPTYANVSTAIDNLVNQWHDNYSGGNTLPARTQYTESMVYSKSQIEAALNVNSKILDGTLGIDFKSISKGEKKVMIAAYKQIFYTVSANLPNNPADVFDKSVTFKELQAKGVSNEAPPLFVSNVAYGRTVFVKLETSSKSNDVEAAFSAALKGTDVKTNGKYSDILENSSFTAVVLGADAAEHNKVVTKDFDVIRNVIKANATFSRKNPAYPISYTSVFLKNNKIAGVNNRSEYVETTSTEYTSGKINLSHQGAYVAQYEILWDEINYDDKGKEVITKRRWDNNWYSKTSPFSTVIPLGANSRNIRIMARECTGLAWEWWRKVIDERDVKLSKEINVNISGSTLSPYGSITYK

SEQ ID NO: 8 - protein, 571 aa, Streptococcus equisimilis
MSNKKIFKKYSRVAGLLTAALIVGNLVTANADSNKQNTANTETTTTNEQPKPESSELTTEKAGQKMDDMLNSNDMIKLAPKEMPLESAEKEEKKSEDNKKSEEDHTEEINDKIYSLNYNELEVLAKNGETIENFVPKEGVKKADKFIVIERKKKNINTTPVDISIIDSVTDRTYPAALQLANKGFTENKPDAVVTKRNPQKIHIDLPGMGDKATVEVNDPTYANVSTAIDNLVNQWHDNYSGGNTLPARTQYTESMVYSKSQIEAALNVNSKILDGTLGIDFKSISKGEKKVMIAAYKQIFYTVSANLPNNPADVFDKSVTFKELQRKGVSNEAPPLFVSNVAYGRTVFVKLETSSKSNDVEAAFSAALKGTDVKTNGKYSDILENSSFTAVVLGGDAAEHNKVVTKDFDVIRNVIKDNATFSRKNPAYPISYTSVFLKNNKIAGVNNRSEYVETTSTEYTSGKINLSHQGAYVAQYEILWDEINYDDKGKEVITKRRWDNNWYSKTSPFSTVIPLGANSRNIRIMARECTGLAWEWWRKVIDERDVKLSKEINVNISGSTLSPYGSITYK

SEQ ID NO: 9 - protein, 571 aa, Streptococcus pyogenes
MSNKKTFKKYSRVAGLLTAALIIGNLVTANAESNKQNTASTETTTTSEQPKPESSELTIEKAGQKMDDMLNSNDMIKLAPKEMPLESAEKEEKKSEDKKKSEEDHTEEINDKIYSLNYNELEVLAKNGETIENFVPKEGVKKADKFIVIERKKKNINTTPVDISIIDSVTDRTYPAALQLANKGFTENKPDAVVTKRNPQKIHIDLPGMGDKATVEVNDPTYANVSTAIDNLVNQWHDNYSGGNTLPARTQYTESMVYSKSQIEAALNVNSKILDGTLGIDFKSISKGEKKVMIAAYKQIFYTVSANLPNNPADVFDKSVTFKDLQRKGVSNEAPPLFVSNVAYGRTVFVKLETSSKSNDVEAAFSAALKGTDVKTNGKYSDILENSSFTAVVLGGDAAEHNKVVTKDFDVIRNVIKDNATFSRKNPAYPISYTSVFLKNNKIAGVNNRTEYVETTSTEYTSGKINLSHQGAYVAQYEILWDEINYDDKGKEVITKRRWDNNWYSKTSPFSTVIPLGANSRNIRIMARECTGLAWEWWRKVIDERDVKLSKEINVNISGSTLSPYGSITYK

SEQ ID NO: 10 - protein, 514 aa, Clostridium novyi
MKKSLKTIIRSISFLSILTLTCSCNFITSTQKNVSLLSGPNKVIKPKKTKSLDDRIYGLKYDPNKILSFNGEKVENFVPNEGFSTPDKYIVIKREKKSISDSTADIAVIDSMNDKTYPGAIQLANRNLIENKPNIVSCERKPITISIDLPGMGEEGKTTITSPTYSSVKAGIDSLLNKWNSHYSSIYSIPTRFSYSDSMVYSKSQLSAKLGCNFKALNKALDIDFDSIYKGQKKVMLLAYKQIFYTVNVDAPNHPSDFFGDKVTFNDLAKKGVNSKNPPVYVSSVSYGRTIYVKLETTSKSANVKAAFKALIENQNISSNSEYKNILNQSSFTATVLGGGAKEHNKVITKNFDEIRNIITNNSEYSPRNPGYPIAYTTSFLKDNSVATVNNKTDYIETTSTEYTNGKITLDHRGAYVAKFNITWDEVSYDKNGKEIVEHKSWEGNDFGRTAHFNTELYLKGNARNICIKAKECTGLAWEWWRTIIDDKNVPLVKNRKVYIWGTTLYPRTLTEIE

SEQ ID NO: 11 - protein, 527 aa, Clostridium tetani
MNKNVLKFVSRSLLIFSMTGLISNYNSSNVLAKGNVEEHSLINNGQVVTSNTKCNLAKDNSSDIDKNIYGLSYDPRKILSYNGEQVENFVPAEGFENPDKFIVVKREKKSISDSTADISIIDSINDRTYPGAIQLANRNLMENKPDIISCERKPITISVDLPGMAEDGKKVVNSPTYSSVNSAINSILDTWNSKYSSKYTIPTRMSYSDTMVYSQSQLSAAVGCNFKALNKALNIDFDSIFKGEKKVMLLAYKQIFYTVSVDPPNRPSDLFGDSVTFDELALKGINNNNPPAYVSNVAYGRTIYVKLETTSKSSHVKAAFKALINNQDISSNAEYKDILNQSSFTATVLGGGAQEHNKIITKDFDEIRNIIKNNSVYSPQNPGYPISYTTTFLKDNSIASVNNKTEYIETTATEYTNGKIVLDHSGAYVAQFQVTWDEVSYDEKGNEIVEHKAWEGNNRDRTAHFNTEIYLKGNARNISVKIRECTGLAWEWWRTIVDVKNIPLAKERTFYIWGTTLYPKTSIETKM

SEQ ID NO: 12 - protein, 528 aa, Listeria ivanovii
MKKIMLLLMTLLLVSLPLAQEAQADASVYSYQGIISHMAPPASPPAKPKTPVEKKNAAQIDQYIQGLDYDKNNILVYDGEAVKNVPPKAGYKEGNQYIVVEKKKKSINQNNADIQVINSLASLTYPGALVKANSELVENQPDVLPVKRDSVTLSIDLPGMVNHDNEIVVQNATKSNINDGVNTLVDRWNNKYSEEYPNISAKIDYDQEMAYSESQLVAKFGAAFKAVNNSLNVNFGAISEGKVQEEVINFKQIYYTVNVNEPTSPSRFFGKSVTKENLQALGVNAENPPAYISSVAYGRDIFVKLSTSSHSTRVKAAFDTAFKGKSVKGDTELENIIQNASFKAVIYGGSAKDEVEIIDGDLSKLRDILKQGANFDKKNPGVPIAYTTNFLKDNQLAVVKNNSEYIETTSKAYSDGKINLDHSGAYVARFNVTWDEVSYDANGNEVVEHKKWSENDKDKLAHFTTSIYLPGNARNINIHAKECTGLAWEWWRTVVDDRNLPLVKNRNVCIWGTTLYPAYSDTVDNPIK

SEQ ID NO: 13 - protein, 529 aa, Listeria monocytogenes
MKKIMLVFITLILVSLPIAQQTEAKDASAFNKENLISSMAPPASPPASPKTPIEKKHADEIDKYIQGLDYNKNNVLVYHGDAVTNVPPRKGYKDGNEYIVVEKKKKSINQNNADIQVVNAISSLTYPGALVKANSELVENQPDVLPVKRDSLTLSIDLPGMTNQDNKIVVKNATKSNVNNAVNTLVERWNEKYAQAYPNVSAKIDYDDEMAYSESQLIAKFGTAFKAVNNSLNVNFGAISEGKMQEEVISFKQIYYNVNVNEPTRPSRFFGKAVTKEQLQALGVNAENPPAYISSVAYGRQVYLKLSTNSHSTKVKAAFDAAVSGKSVSGDVELTNIIKNSSFKAVIYGGSAKDEVQIIDGNLGDLRDILKKGATFNRETPGVPIAYTTNFLKDNELAVIKNNSEYIETTSKAYTDGKINIDHSGGYVAQFNISWDEINYDPEGNEIVQHKNWSENNKSKLAHFTSSIYLPGNARNINVYAKECTGLAWEWWRTVIDDRNLPLVKNRNISIWGTTLYPKYSNSVDNPIE

SEQ ID NO: 14 - protein, 530 aa, Listeria seeligeri
MKIFGLVIMSLLFVSLPITQQPEARDVPAYDRSEVTISPAETPESPPATPKTPVEKKHAEEINKYIWGLNYDKNSILVYQGEAVTNVPPKKGYKDGSEYIVVEKKKKGINQNNADISVINAISSLTYPGALVKANRELVENQPNVLPVKRDSLTLSVDLPGMTKKDNKIFVKNPTKSNVNNAVNTLVERWNDKYSKAYPNINAKIDYSDEMAYSESQLIAKFGTAFKAVNNSLNVNFEAISDGKVQEEVISFKQIYYNINVNEPTSPSKFFGGSVTKEQLDALGVNAENPPAYISSVAYGRQVYVKLSSSSHSNKVKTAFEAAMSGKSVKGDVELTNIIKNSSFKAVIYGGSAKEEVEIIDGNLGELRDILKKGSTYDRENPGVPISYTTNFLKDNDLAVVKNNSEYIETTSKSYTDGKINIDHSGGYVAQFNISWDEVSYDENGNEIKVHKKWGENYKSKLAHFTSSIYLPGNARNINIYARECTGLFWEWWRTVIDDRNLPLVKNRNVSIWGTTLYPRHSNNVDNPIQ

SEQ ID NO: 15 - protein, 497 aa, Streptococcus suis
MRKSSHLILSSIVSLALVGVTPLSVLADSKQDINQYFQSLTYEPQEILTNEGEYIDNPPATTGMLENGRFVVLRREKKNITNNSADIAVIDAKAANIYPGALLRADQNLLDNNPTLISIARGDLTLSLNLPGLANGDSHTVVNSPTRSTVRTGVNNLLSKWNNTYAGEYGNTQAELQYDETMAYSMSQLKTKFGTSFEKIAVPLDINFDAVNSGEKQVQIVNFKQIYYTVSVDEPESPSKLFAEGTTVEDLKRNGITDEVPPVYVSSVSYGRSMFIKLETSSRSTQVQAAFKAAIKGVDISGNAEYQDILKNTSFSAYIFGGDAGSAATVVSGNIETLKKIIEEGARYGKLNPGVPISYSTNFVKDNRPAQILSNSEYIETTSTVHNSSALTLDHSGAYVAKYNITWEEVSYNEAGEEVWEPKAWDKNGVNLTSHWSETIQIPGNARNLHVNIQECTGLAWEWWRTVYDKDLPLVGQRKITIWGTTLYPQYADEVIE

SEQ ID NO: 16 - protein, 466 aa, Streptococcus mitis
MANKAVNDFILAMDYDKKKLLTHQGESIENRFIKEGNQLPDEFVVIERKKRSLSTNTSDISVTATNDSRLYPGALLVVDETLLENNPTLLAVDRAPMTYSIDLPGLASSDSFLQVEDPSNSSVRGAVNDLLAKWHQDYGQVNNVPARMQYEKITAHSMEQLKVKFGSDFEKTGNSLDIDFNSVHSGEKQIQIVNFKQIYYTVSVDAVKNPGDVFQDTVTVEDLRQRGISADRPLVYISSVAYGRQVYLKLETTSKSDEVEAAFEALIKGVKVAPQTEWKQILDNTEVKAVILGGDPSSGARVVTGKVDMVEDLIQEGSRFTADHPGLPISYTTSFLRDNVVATFQNSTDYVETKVTAYRNGDLLLDHSGAYVAQYYITWDELSYDYQGKEVLTPKAWNRNGQDLTAHFTTSIPLKGNVRNLSVKIRECTGLAWEWWRTVYEKNDLPLVRKRTISIWGTTLYPQVED

SEQ ID NO: 17 - protein, 532 aa, Streptococcus intermedius
MKTKQNIARKLSRVVLLSTLVLSSAAPISAAFAETPTKPKAAQTEKKPEKKPENSNSEAAKKALNDYIWGLQYDKLNILTHQGEKLKNHSSREAFHRPGEYVVIEKKKQSISNATSKLSVSSANDDRIFPGALLKADQSLLENLPTLIPVNRGKTTISVNLPGLKNGESNLTVENPSNSTVRTAVNNLVEKWIQKYSKTHAVPARMQYESISAQSMSQLQAKFGADFSKVGAPLNVDFSSVHKGEKQVFIANFRQVYYTASVDSPNSPSALFGSGITPTDLINRGVNSKTPPVYVSNVSYGRAMYVKFETTSKSTKVQAAIDAVVKGAKLKAGTEYENILKNTKITAVVLGGNPGEASKVITGNIDTLKDLIQKGSNFSAQSPAVPISYTTSFVKDNSIATIQNNTDYIETKVTSYKDGALTLNHDGAFVARFYVYWEELGHDADGYETIRSRSWSGNGYNRGAHYSTTLRFKGNVRNIRVKVLGATGLAWEPWRLIYSKNDLPLVPQRNISTWGTTLHPQFEDKVVKDNTD

SEQ ID NO: 18 - protein, 665 aa, Streptococcus mitis
MNQEKRLHRFVKKCGLGVCSAVVAAFLLNAQGVALATEQGNRPVETENIARGKQASQSSTAYGGAATRAVDGNVDSDYGHHSVTHTNFEDNAWWQVDLGKTENVGKVKLYNRGDGNVANRLSNFDVVLLNEAKQEVARQHFDSLNGKAELEVFFTAKDARYVKVELKTKNTPLSLAEVEVFRSATTQVGQDRTAPVVDQTSALKDYLFGLTYNPLDILTRKGETLENRYNTSAKEQNGEFVVVEKIKKTLSTGTADVSINGNQNVFLGGLYKANQNLLENQPELISLARAKGTVSVDLPGMIHSENKIEANPTTSGMQEAMNTLVEKWTKNYSSSHSVPARVQYESTTAYSMNQLKAKFGADFEKAGAPLKIDFEAVQKGEKQIEVVNFKQIYYTATFDAPTNPAAVFDKSVTPEDLKQRGVDSQTPPVYVSNVSYGRQIYVKFESTSKSTELKAAINAVIKGATIAPNSEWSRLLKNTSVTAVIVGGNASGAAKVVTGTVENLKELIREGANFSAQSPAVPISYKTAFLKDNAQATLQNSTDYIETKVTSYKNGFLKLHHKGAYIARYYIYWDEITYDEQGNPEIRSRQWEDNGKNRTSGFQTEIQFRGNVRNLRIKVQEKTGLVWEPWRTVYNRTDLPLVQQRTITHWGTTLNPKVDEKIVNE

SEQ ID NO: 19 - protein, 534 aa, Arcanobacterium pyogenes
MKRKAFASLVASVVAAATVTMPTASFAAGLGNSSGLTDGLSAPRASISPTDKVDLKSAQETDETGVDKYIRGLKYDPSGVLAVKGESIENVPVTKDQLKDGTYTVFKHERKSFNNLRSDISAFDANNAHVYPGALVLANKDLAKGSPTSIGIARAPQTVSVDLPGLVDGKNKVVINNPTKSSVTQGLNGLLDGWIQRNSKYPDHAAKISYDETMVTSKRQLEAKLGLGFEKVSAKLNVDFDAIHKRERQVAIASFKQIYYTASVDTPTSPHSVFGPNVTAQDLKDRGVNNKNPLGYISSVSYGRQIFVKLETTSTSNDVQAAFSGLFKAKFGNLSTEFKAKYADILNKTRATVYAVGGSARGGVEVATGNIDALKKIIKEESTYSTKVPAVPVSYAVNFLKDNQLAAVRSSGDYIETTATTYKSGEITFRHGGGYVAKFRLKWDEISYDPQGKEIRTPKTWSGNWAARTLGFRETIQLPANARNIHVEAGEATGLAWDPWWTVINKKNLPLVPHREIVLKGTTLNPWVEDNVKS

SEQ ID NO: 20 - DNA, 1416 bp, Streptococcus pneumoniae
ctagtcattttctaccttatcctctacctgaggatagagagttgttccccaaatagaaatcgtccgcttacgcactagtggcaaatcggttttttcataaaccgtacgccaccattcccaggcaagcccggtacactctctaattttgacagagagattacgaacattcccttttaaaggaatactagtggtaaagtgagccgtcaaatcctgcccatttctgtcccaagccttaggagtcaagacttccttaccttgatgatcataggataattcatcccaagtaatataatattgggcaacataggcaccactatgatccagcagtaaatctccgtttctgtaagctgtaaccttagtctcaacatagtctgtactgttttgaaaggtcgcaactacattgtcacgtaaaaaagaagttgtataggaaatcggcaagcctggatgatctgctgtaaagcgactgccttcttgaatcaagtcctctaccatatccaccttgcctgttacaactcgggcacccgaacttgggtcgccccctaaaataaccgccttcacttctgtattgtccaaaatctgcttccactctgtctgaggagctaccttgactccttttatcaaagcttcaaaagcagcctctacttcatcactcttactcgtggtttccaacttgagatagacttggcgcccataagcaacactcgaaatatagaccaaaggacgctctgcagaaattcctctctgttttaaatcctctaccgttacagtatcttgaaacacatctcctggatttttaacagcgtctacgctgactgtataataaatctgcttaaaattaacaatctgaatctgcttttcacctgaatggacagagttaaaatcaatatcaagagaattccctgtcttttcaaagtcagaaccaaacttgaccttgagttgttccatgctgtgagccgttattttttcatactgcattctagctgggacattattgacctgaccataatcttgatgccacttagccaacaaatcgtttaccgctccgcgaacacttgaattgctggggtcttccacttggagaaagctatcgctacttgccaaaccaggcaaatcaatactataagtcatcggagcacgatcaaccgcaagaagagtgggattattctctaacaaggtctcatccactacgagaagtgctccaggatagaggcgactgtcgttggtagctgttacagaaatatcacttgtatttgtcgacaagctccgcttctttctttcgataacaacaaactcatcgggtagctgattaccctctttgatgaaacgattttcaatactttctccctgatgggtcaagagtttctttttatcgtaattcatagctagtataaagtcatttactgctttatttgccat

SEQ ID NO: 21 - DNA, 1530 bp, Bacillus cereus
ctgaatattaagaaaaacactaaaagaagaaagttccttgcatgtttattagttagtttatgcactattaattattcatctatttccttcgcagaaacacaagcaagtaatgcaactgatgtaaccaaaaatgctagtggcattgatactggtatagcaaatcttaaatataataatcaagaggttttagctgtaaatggtgataaagtagaaagttttgttccgaaagaaagtatcaattcaaatggtaaatttgtagtagtggaacgcgagaaaaaatcacttacaacgtcaccagtcgatatttcaattattgattctgtagtgaatcgcacgtatccaggagctgtacaacttgcaaataaagcttttgcagacaatcaaccaagtttattagtggctaagagaaagcctttgaatattagtatagacttaccgggcatgagaaaagaaaatacaatcactgtccaaaatccgacatatggtaatgtagctggagcagtagacgatttagtatctacttggaatgaaaagtattctacaacacatacgttacctgcaagaatgcagtatacggaatctatggtttatagtaaatcacaaatagcaagtgctcttaatgttaacgctaaatatcttgataacagtctaaacattgattttaatgcggttgcaaatggagagaaaaaagtgatggtagcggcgtataagcaaatattttatacggtaagtgctgaactacctaacaatccatccgacctttttgataatagcgttacttttgacgagttaactcgaaaaggcgtaagtaattcggctccacctgttatggtttcaaatgtagcttatggtagaacgatttatgtaaaattagaaacaacatctaagagcaaagatgtacaagctgcttttaaagccttacttaagaataacagcgttgaaacaagtggacagtataaagatatttttgaagaaagtacctttactgctgtagtattaggcggagatgcgaaagagcataacaaggttgttactaaagatttcaatgaaatccgaaatatcattaaagataatgctgaattaagtcttaaaaatccagcatacccaatttcatatacaagcactttcttaaaagataattcaactgctgctgttcataacaatacagattatattgagacgacaactacagaatattcaagtgctaaaatgacacttgatcattacggtgcttacgttgctcaatttgatgtatcttgggatgaattcacatttgaccaaaagggtaacgaagtactaacacataaaacgtgggatggtagcggaaaagacaaaacggctcattactctacagttatcccactcccaccaaattcaaaaaatataaaaattgtagcaagagaatgtacaggtcttgcatgggaatggtggagaacaattattaatgaacaaaatgttccattaacaaatgaaataaaagtttcaattggaggaacaacattatacccaacagctagtattagtcattaa

SEQ ID NO: 22 - DNA, 1539 bp, Bacillus anthracis
ctaatgactaatagtagcagttggatataatgttgttcctccaattgaaacctttatttcatttgttaatggaacattttgttcattaatgatagttctccaccattcccatgcaagacctgtacattctcttgcaacgatttttatattttttgaatttggtggaagagggataactgtagagtaatgggctgttttgtctttgccactaccttcccatgttttatgtgttagtacttctttcccattttgatcaaatgtaaattcatcccaagatacatcaaattgagcaacgtaagcaccgtaatgatcgagtgtcattttagcacttgaatattctgtagttgtcgtctcgatataatctgtattgttatgaacagcagcagttgcattatcttttaagaacgtgcttgtatatgaaattgggtatgctggatttttaaagcttaattcagcattatctttaataatatttcggatttcattgaaatcttttgtaacaaccttgttatgctctttcgcatctccgcctaatactacagcagtaaaggtactttcttcaaaaatatctttgtactgtccactcgtttcgacgctgttattcttaagtagagctttaaatgcagcttgtacatctttactcttagatgttgtttctaattttacataaaccgttctaccataagctacatttgaaaccataacaggtggagccgaattacttactcctttacgagttaactcatcaaaagtaacactattatcaaagagatcagatggattattaggtagttcagcacttacagtataaaatatttgtttatatgccgccaccatcactttcttttctccatttgcaactgcattaaagtcaatatttagactgttatcaagatatttagcattaacattaagagcacttgcgatttgtgatttactataaaccatagattctgtatactgcattcttgcaggtaacgtatgtgttgtggaatacttttcattccaagtagatactaaatcatctactgctccagccacattaccatatgtcggattttggacagtgattgtattttcttttctcatgccaggtaagtctatactaatattcaaaggctttctcttagctactaataaactcggttgattgtctgcaaatgctttattggcaagttgtacagctcctggatacgtacgattcactacagaatcaataatcaaaatatcgactggtgacgttgtaagtgattttttctcgcgttccactactacaaatttaccgtttgaattgatactctctttcggaataaaactctctactttatcaccatttactgctaaaatatctctactatcatactttagatttgctataccagtattaatatcactagcattttttattgcaccagttgcattaccggcttgtgtttctgcaaaagaaatagacgaataatgaatggtacatagactaactaataaacatgcaaggaactttcttcttttagtgtttttcttaatattcagaaaaatcac

SEQ ID NO: 23 - DNA, 1530 bp, Bacillus thuringiensis
ctgaatattaagaaaaacactaaaagaagaaagttccttgcatgtttattagttagtctatgcaccattaattattcatctatttccttcgcagaaacacaagcaagtaatgcgactgatgtaaccaaaaatgctagtggcattgatactggtatagcaaatcttaaatataatattcaagaggttttagctgtaaatggtgataaagtagaaagttttgttccgaaagaaagtatcaattcaaatggtaaatttgtagtagtggaacgcgagaaaaaatcacttacaacgtcaccagtcgatatttcaattattgattctgtggtgaatcgcacgtatccaggagctgtacaacttgctaataaagcttttgcagacaatcaaccgagtttattagtggctaagagaaagcctttgaatattagtatagacttaccgggcatgagaaaagaaaatacaatcactgtccaaaatccgacatatggtaatgtagctggagcagtagacgatttagtatctacttggaatgaaaagtattctacaacacatacgttacctgcaagaatgcagtatacggaatctatggtttatagtaaatcacaaattgcaagtgctcttaatgttaacgctaaatatcttgataacagtctaaatattggttttaatgcggttgcaaatggagagaaaaaagtgatggtagcggcgtataagcaaatattttatacggtaagtgctgaactacctaacaatccatccgacctttttgataatagcgttacttttgacgagttaactcgaaaaggcgtaaataattcggctccacctgttatggtttcaaatgtagcttatggtagaacgatttatgtaaaattagaaacaacatctaagagcaaagatgtacaagctgcttttaaagccttacttaagaataacagcgttgaaacaagtggacagtataaagatatttttgaagaaagtacctttactgctgtagtattaggcggagatgcgaaagaacataacaaggttgttactaaagatttcaatgaaatccgaaatattattaaagataatgctgaattaagtcttaaaaatccagcatacccaatttcatatacaagtactttcttaaaagataatgcaactgctgctgttcataacaatacagattatattgagacgacaactacagaatattcaagtgctaaaatgacacttgatcattacggtgcttacgttgctcaatttgatgtatcttgggatgaattcacatttgatcaaaagggtaacgaagtactaacacataaaacgtgggatggtagtggaaaagacaaaacggctcattactctacagttatccctcttccaccgaattcaaaaaatataaaaattgtagcaagagaatgtacaggtcttgcatgggaatggtggagaacaattattaatgaacaaaacgttccattaacaaatgaaataaaagtttcaattggaggaacaacattatacccaacagctagtattagtcattaa

SEQ ID NO: 24 - DNA, 1503 bp, Clostridium perfringens
atgataagatttaagaaaacaaaattaatagcaagtattgcaatggctttatgtctgttttctcaaccagtaatcagtttctcaaaggatataacagataaaaatcaaagtattgattctggaatatcaagtttaagttacaatagaaatgaagttttagctagtaatggagataaaattgaaagctttgttccaaaggaaggtaaaaaagctggtaataaatttatagttgtagaacgtcaaaaaagatcccttacaacatcaccagtagatatatcaataattgattctgtaaatgaccgtacatatccaggagcattacaacttgcagataaagcatttgtggaaaatagacctacaatcttaatggtaaaaagaaagcctattaacattaatatagatttaccaggattaaagggcgaaaatagtataaaggttgatgatccaacctatggaaaagtttctggagcaattgatgaattagtatctaagtggaatgaaaagtattcatctacacatactttaccagcaagaactcaatattcagaatctatggtttatagtaaatcacaaatatcaagtgcccttaatgttaatgctaaagtccttgaaaactcacttggagtagactttaatgcagtagcaaacaatgagaaaaaagttatgattttagcatataaacaaatattctatacagtaagtgcagatttacctaagaatccatcagatctttttgatgacagtgttacatttaatgatttaaaacaaaagggagtaagtaatgaagcacctccacttatggtttcaaatgtagcttatggaagaacaatatatgttaagttagaaactacttctagtagtaaagatgtacaagctgctttcaaagctcttataaagaacactgatataaaaaatagtcaacaatataaagatatttatgaaaatagttccttcacagcagtagttttaggaggagatgcacaagaacataacaaagttgtaactaaagactttgatgaaataagaaaagtaattaaagacaatgcaacttttagtacaaaaaacccagcatatccaatatcttatactagtgttttcttaaaagataactcagttgctgctgttcacaataaaacagattatatagaaacaacttctacagagtattctaagggaaaaataaacttagatcatagtggagcctatgttgcacagtttgaagtagcctgggatgaagtttcatatgacaaagaaggaaatgaagttttaactcataaaacatgggatggaaattatcaagataaaacagctcactattcaacagtaatacctcttgaagctaatgcaagaaatataagaataaaagcaagagagtgtacaggccttgcttgggaatggtggagagatgttataagtgaatatgatgttccattaacaaataatataaatgtttcaatatggggaacaactttataccctggatctagtattacttacaattaa

SEQ ID NO: 25 - DNA, 1506 bp, Bacillus alvei
atgaagaaaaaatcaaaccacttgaaaggaaggaaagtactcgtaagtttgttagtaagcttacaagtgttcgcttttgcgagtatttcctccgcagcaccaaccgaacccaatgatattgatatggggatcgcaggactgaactataatcgcaatgaggttttggctattcaaggggatcaaatcagtagttttgttcccaaagaaggcattcagtccaatggcaaatttatcgtggttgaacgggacaaaaaatcactcacaacgtcacccgtagatatttccatcgttgattcaatcacgaatcgcacgtatccaggcgcaatacagcttgcaaataaggattttgccgataatcagcctagtctggttatggctgcgagaaaaccattagatattagcatcgatctgcctggtttgaagaacgagaatacaatttccgttcaaaatccaaattacggcactgtatctagtgccattgatcagctcgtgtcgacttggggcgagaagtattccagcacgcatacactgcctgcaagattacaatacgctgaatccatggtttacagccaaaatcaaatttccagcgccctgaatgtgaacgctaaagtactgaacggtacactcggaatcgactttaacgcggttgcaaatggcgagaaaaaagtgatggttgctgcttacaagcaaatcttttataccgtaagtgcaggactgcccaacaatccatcagacttgttcgatgacagtgtgacatttgctgagttagctcgcaagggagtaagcaatgaggcaccgccgctgatggtatctaacgtggcttacggcagaactatttacgtaaaattggaaacaacttctaagagcaatgacgtacaaacggcatttaaattgttgctcaataatcctagcatacaagctagcggacagtacaaagatatttatgagaacagctcgtttactgccgttgtactaggcggcgacgcgcaaacccataaccaagtcgttacgaaagacttcaatgttatccaaagtgtaatcaaggacaatgcacaatttagcagcaagaaccctgcttacccgatttcatatacaagtgtcttcttgaaagacaattccattgctgctgttcacaacaataccgagtatatcgagacgaaaacgacggaatattcgaagggtaaaattaagcttgatcatagtggtgcatatgtagctcagtttgaagtatattgggatgaattttcatatgatgcagatggacaagaaatcgtgactcgtaaaagttgggatggaaattggcgcgatagatctgctcatttctcaacagaaatcccacttcctcctaatgccaagaacataagaatttttgcgagagaatgcacaggtcttgcttgggaatggtggagaacagttgttgatgaatataacgttccgttagcaagcgatattaatgtttcgatttggggaacaacgttatatccgaaatcatccattactcactaa

SEQ ID NO: 26 - DNA, 1725 bp, Streptococcus canis
atgaaggacatgtctaataaaaaaatatttaaaaaatacagtcgcgtcgctgggctattaacggcagctcttatcgttggtaatcttgttactgctaatgctgactcgaacaaacaaaacactgccaatacagaaaccacaacgacaaatgaacaaccaaaaccagaaagtagtgagctaactacagaaaaagcaggtcagaaaatggatgatatgcttaactctaacgatatgattaagcttgctcccaaagaaatgccactagaatctgcagaaaaagaagaaaaaaagtcagaagacaataaaaaaagcgaagaagatcatactgaagaaatcaatgacaagatttattcactaaattataatgagcttgaagtacttgctaaaaatggtgaaaccattgaaaactttgttcctaaagaaggcgttaagaaagctgacaaatttattgtcattgaaagaaagaaaaaaaatatcaacactacaccggtcgatatttccatcattgactctgtcactgataggacctatccagcagcccttcagctggctaataaaggttttaccgaaaacaaaccagacgcagtagtcaccaagcgaaacccacaaaaaatccatattgatttaccaggtatgggagacaaagcaacggttgaggtcaatgaccctacctatgccaatgtttcaacagctattgataatcttgttaaccaatggcatgataattattctggtggtaatacgcttcctgccagaacacaatatactgaatcaatggtatattctaaatcacagattgaagcagctctaaatgttaatagtaaaatcttagatggtactttaggcattgatttcaagtcgatttcaaaaggtgaaaagaaggtgatgattgcagcatacaagcaaattttttacaccgtatcagcaaaccttcctaataatcctgcggatgtgtttgataaatcagtgacctttaaagagttgcaagcaaaaggtgtcagcaatgaagccccgccactctttgtgagtaacgtagcttatggtcgaactgtttttgtcaaactagaaacaagttctaaaagtaatgatgttgaagcggcctttagtgcagctctaaaaggaacagatgttaaaactaatggaaaatactctgatattttagaaaatagttcatttacagctgtcgttttaggagcagatgctgcagagcacaataaggtagtcacaaaagactttgatgttattagaaacgttatcaaagctaatgctaccttcagtagaaaaaacccagcttatcctatttcatacaccagtgttttccttaaaaataataaaattgcgggtgtcaataacagaagtgaatacgttgaaacaacatctaccgagtacacgagtggaaaaattaacctgtctcatcaaggtgcctatgttgctcaatatgaaatcctttgggatgaaatcaattatgatgacaaaggaaaagaagtgattactaaacgacgttgggacaacaactggtatagtaagacatcaccatttagcacagttatcccactaggagctaattcacgaaatatccgtatcatggctagagagtgcaccggcttagcttgggaatggtggcgaaaagtgatcgacgaaagagatgtgaaactgtctaaagaaatcaatgtcaacatctcaggatcaaccctgagcccatatggttcgattacttataagtag

SEQ ID NO: 27 - DNA, 1715 bp, Streptococcus equisimilis
atgtctaataaaaaaatatttaaaaaatacagtcgcgtcgctgggctattaacggcagctcttatcgttggtaatcttgttactgctaatctgactcgaacaaacaaaacactgccaatacagaaaccacaacgacaaatgaacaaccaaaaccagaaagtagtgagctaactacagaaaaagcaggtcagaaaatggatgatatgcttaactctaacgatatgattaagcttgctcccaaagaaatgccactagaatctgcagaaaaagaagaaaaaaagtcagaagacaataaaaaaagcgaagaagatcatactgaagaaatcaatgacaagatttattcactaaattataatgagcttgaagtacttgctaaaaatggtgaaaccattgaaaactttgttcctaaagaaggcgttaagaaagctgacaaatttattgtcattgaaagaaagaaaaaaaatatcaacactacaccggtcgatatttccatcattgactctgtcactgataggacctatccagcagcccttcagctggctaataaaggttttaccgaaaacaaaccagacgcagtagtcaccaagcgaaacccacaaaaaatccatattgatttaccaggtatgggagataaagcaacggttgaggtcaatgaccctacctatgccaatgtttcaacagctattgataatcttgttaaccaatggcatgataattattctggtggtaatacgcttcctgccagaacacaatatactgaatcaatggtatattctaaatcacagattgaagcagctctaaatgttaatagtaaaatcttagatggtactttaggcattgatttcaagtcgatttcaaaaggtgaaaagaaggtgatgattgcagcatacaagcaaattttttacaccgtatcagcaaaccttcctaataatcctgcggatgtgtttgataaatcagtgacctttaaagagttgcaacgaaaaggtgtcagcaatgaagccccgccactctttgtgagtaacgtagcttatggtcgaactgtttttgtcaaactagaaacaagttctaaaagtaatgatgttgaagcggcctttagtgcagctctaaaaggaacagatgttaaaactaatggaaaatactctgatattttagaaaatagttcatttacagctgtcgttttaggaggagatgctgcagagcacaataaggtagtcacaaaagactttgatgttattagaaacgttatcaaagataatgctacattcagtagaaaaaacccagcttatcctatttcatacaccagtgttttccttaaaaataataaaattgcgggtgtcaataacagaagtgaatacgttgaaacaacatctaccgagtacacgagtggaaaaattaacctgtctcatcaaggtgcctatgttgctcaatatgaaatcctttgggatgaaatcaattatgatgacaaaggaaaagaagtgattacaaaacgacgttgggacaacaactggtatagtaagacatcaccatttagcacagttatcccactaggagctaattcacgaaatatccgtatcatggctagagagtgcaccggattagcttgggaatggtggcgaaaagtgatcgacgaaagagatgtgaaactgtctaaagaaatcaatgtcaacatctcaggatcaaccttgagcccatatggttcgattacttataagtag

SEQ ID NO: 28 - DNA, 1716 bp, Streptococcus pyogenes
atgtctaataaaaaaacatttaaaaaatacagtcgcgtcgctgggctactaacggcagctcttatcattggtaatcttgttactgctaatgctgaatcgaacaaacaaaacactgctagtacagaaaccacaacgacaagtgagcaaccaaaaccagaaagtagtgagctaactatcgaaaaagcaggtcagaaaatggatgatatgcttaactctaacgatatgattaagcttgctcccaaagaaatgccactagaatctgcagaaaaagaagaaaaaaagtcagaagacaaaaaaaagagcgaagaagatcacactgaagaaatcaatgacaagatttattcactaaattataatgagcttgaagtacttgctaaaaatggtgaaaccattgaaaattttgttcctaaagaaggcgttaagaaagctgataaatttattgtcattgaaagaaagaaaaaaaatatcaacactacaccagtcgatatttccattattgactctgtcactgataggacctatccagcagcccttcagctggctaataaaggttttaccgaaaacaaaccagacgcggtagtcaccaagcgaaacccacaaaaaatccatattgatttaccaggtatgggagacaaagcaacggttgaggtcaatgaccctacctatgccaatgtttcaacagctattgataatcttgttaaccaatggcatgataattattctggtggtaatacgcttcctgccagaacacaatatactgaatcaatggtatattctaagtcacagattgaagcagctctaaatgttaatagcaaaatcttagatggtactttaggcattgatttcaagtcgatttcaaaaggtgaaaagaaggtgatgattgcagcatacaagcaaattttttacaccgtatcagcaaaccttcctaataatcctgcggatgtgtttgataaatcagtgacctttaaagatttgcaacgaaaaggtgtcagcaatgaagctccgccactctttgtgagtaacgtagcctatggtcgaactgtttttgtcaaactagaaacaagttctaaaagtaatgatgttgaagcggcctttagtgcagctctaaaaggaacagatgttaaaacgaatggaaaatactctgatatcttagaaaatagctcatttacagctgtcgttttaggaggagatgctgcagagcacaataaggtggtcacaaaagactttgatgttattagaaacgttatcaaagacaatgctaccttcagtagaaaaaacccagcttatcctatttcatacaccagtgttttccttaaaaataataaaattgcgggtgtcaataacagaactgaatacgttgaaacaacatctaccgagtacactagtggaaaaattaacctgtctcatcaaggcgcgtatgttgctcaatatgaaatcctttgggatgaaatcaattatgatgacaaaggaaaagaagtgattacaaaacgacgttgggacaacaactggtatagtaagacatcaccatttagcacagttatcccactaggagctaattcacgaaatatccgtatcatggctagagagtgcaccggcttagcttgggaatggtggcgaaaagtgatcgacgaaagagatgtgaaactatctaaagaaatcaatgtcaacatctcaggatcaaccttgagcccatatggttcgattacttataagtag

SEQ ID NO: 29 - DNA, 1545 bp, Clostridium novyi
atgaagaaatctttaaaaactataattcgtagcatatcttttctctcaatattaacattaacttgtagttgcaactttataacaagcacccagaaaaatgtaagcttattatcgggacctaataaagttattaaacctaagaaaactaaatccttagatgataggatttatggattaaaatatgatcctaataaaatactatcatttaatggagaaaaagttgaaaattttgtacctaacgaaggtttttcaacacccgataagtacatcgttataaaacgtgaaaagaaaagtatatcagattctacagcagatatagctgttatagactcgatgaatgacaaaacttatcctggtgcaatacaacttgcaaatagaaatcttatagaaaacaagcctaatatagtatcttgtgaaagaaagccaataacaataagtatagatttacctgggatgggtgaagaagggaagacaactataacttctcctacttattcttctgttaaagcaggaattgattcattgctaaataagtggaattcacattattcgtcaatatatagcattccaactagatttagctattcagattctatggtttatagtaagtctcaattatcagctaaattaggttgtaatttcaaagctttaaataaagcattggatattgattttgattctatttataaaggacaaaagaaagtaatgcttcttgcatataagcaaattttttatacagtaaatgtagatgccccaaatcatccatcagacttctttggggataaagtaacatttaatgacttagcaaaaaaaggagttaatagtaagaatcctcctgtatacgtttcaagtgtatcttatggtagaactatttatgtaaaacttgaaactacttctaaaagtgccaatgtaaaagctgcatttaaagcactaatagaaaatcaaaatataagcagtaattctgagtacaaaaatattttaaatcaaagctcatttacagctacagtattaggtggtggagctaaagaacataacaaagtaataactaaaaactttgatgaaataagaaatataataactaacaactcagaatatagtcctagaaatccaggttatcctatagcatatactacttcttttctaaaagataatagtgttgcaacagtgaacaataaaacagattatatagagacaacctctacagaatatactaatggaaaaattactcttgatcatagaggtgcatatgtagctaaattcaatattacttgggatgaagtaagctatgataagaatggaaaagaaatagtagaacacaaatcatgggaaggaaatgacttcggtagaacagctcatttcaatacagaattatacctaaaaggtaacgctcgaaatatttgcataaaagctaaagaatgcactggtcttgcttgggaatggtggagaactataatagatgataaaaatgttcctttagttaaaaacagaaaagtctatatttggggaacaacattatatcctagaacattaacagaaatagaataa

SEQ ID NO: 30 - DNA, 1584 bp, Clostridium tetani
ttacattttagtttcaattgatgtctttggatataatgttgtaccccatatatagaaagttctttcttttgctagtggtatatttttaacatctacaatggttctccaccattcccatgcaagacctgtacattctcttatttttacagatatatttcgtgcatttccttttaaatatatttctgtattaaaatgagccgttctatctctattatttccttcccaagctttatgttcaactatttcatttcccttttcgtcatagctaacctcatcccatgttacttggaattgagcaacatacgctccactatgatcaagtactattttaccattagtatattctgttgcagttgtttctatatattctgttttattatttacggatgctatactattgtcttttaaaaatgtagtagtatatgaaattggatatcctggattttgtggactatacactgaattatttttaataatatttcttatttcatcaaaatccttagtgattatcttattatgttcttgtgctcctccccctaaaacagtagctgtaaatgaactttgatttaatatatccttatattctgcattactacttatatcctggttattgattagtgctttaaaagctgctttaacatgtgaactcttagaggtagtttcaagttttacataaattgttctaccatatgcaacatttgaaacatatgcaggaggattattattatttatcccctttaaagccaattcatcaaaagttacactatcaccaaataaatctgatggacgatttggtgggtctacacttactgtataaaaaatttgtttgtatgcaagaagcataacctttttttcacctttaaatatggaatcaaaatctatatttaatgctttgtttaaagctttaaaattgcatccaactgctgcagataactgtgattggctatacaccatagtatcagaataactcattcttgtaggtatagtatatttagatgaatactttgaattccatgtatctaatatagaatttattgcagaattaactgaggagtaggtaggtgaattaacaactttcttaccatcttcagccatacccggtaagtcaacacttatagtaataggttttctctcacatgaaattatatcaggtttgttttccataagatttctgttagcaagttgtatagctccaggataagttctatcatttattgagtctataattgaaatgtctgctgtggaatctgaaatactcttcttctcacgttttaccacaatgaacttatctggattttcaaatccttcagcaggtacaaaattttctacctgttcaccattatatgataatatcttacgtggatcataggataatccataaatatttttgtctatgtcactactgttgtcttttgccaaattacattttgtatttgacgttactacttgtccattattgattaatgaatgttcctctacatttcctttagctaatacattactggaattataattagatattaagccagtcattgaaaatattagcaatgaacgtgatacaaattttaatacatttttgttcat

SEQ ID NO: 31 - DNA, 1587 bp, Listeria ivanovii
atgaaaaaaataatgctacttttaatgacattgttactagtaagtttaccgttagcacaagaagctcaagcagatgcctcagtatatagttaccaaggcataatttcacacatggcaccaccagcgtctccgcctgcaaagcctaagacgccggttgaaaagaaaaatgcagctcaaatcgatcaatatatacaagggctggattatgataaaaacaatatattagtgtacgatggagaagctgttaaaaatgttccaccaaaagcaggatacaaagaaggaaatcaatatattgtagtggagaaaaagaaaaaatctatcaatcaaaataacgcagatattcaagttattaactcgcttgcaagccttacttatccaggagctttagtgaaggcgaattcagagttagtcgaaaatcaacccgatgtcctccctgtgaaacgagattcagttacacttagtattgatttgcctggaatggttaaccatgacaatgaaatagtcgttcaaaatgcaactaaatccaatataaatgacggagtgaatactttagtagatcgttggaataataaatactccgaagaatacccaaatattagtgcgaaaattgactatgatcaagaaatggcctatagcgaatcgcaattagttgcaaaatttggtgcagcatttaaagctgttaataatagtttgaatgtaaactttggagcgattagtgaaggtaaggtgcaagaagaagttattaatttcaaacaaatttattatactgttaatgttaatgaacctacaagcccttccagattctttggtaaaagtgttactaaagaaaacttgcaagcgctgggcgtaaatgcggaaaatccacccgcatacatctctagtgttgcatatggtcgtgacattttcgtgaaattatcgactagttcacacagcaccagagtgaaggctgcattcgatactgcatttaagggtaaatcagttaaaggtgatacagaattagaaaatattattcaaaatgcttcatttaaagcggtgatttatggtggttcagccaaagatgaagtagaaataattgatggagatttaagcaaattacgagatattttaaaacaaggggctaattttgataagaaaaatccgggcgtaccgattgcgtatacaactaatttcttgaaagataatcagttagcagttgttaaaaataattcggaatatatcgaaacaacttctaaggcttactcggatggaaaaattaacctagatcattccggtgcctatgttgcgagattcaatgttacttgggatgaagttagctatgatgctaatggaaatgaagttgttgaacataaaaaatggtccgaaaatgataaagataagttagctcattttacgacatcaatctatttgccagggaatgcaaggaatattaatattcatgcgaaagaatgtactggcttggcttgggaatggtggagaacggttgtggatgatagaaacttgccattagtaaaaaatagaaatgtttgtatctggggaacaacgctttatccagcgtatagtgatactgtagataatccaattaagtaa

SEQ ID NO: 32 - DNA, 1590 bp, Listeria monocytogenes
atgaaaaaaataatgctagtttttattacacttatattagttagtctaccaattgcgcaacaaactgaagcaaaggatgcatctgcattcaataaagaaaatttaatttcatccatggcaccaccagcatctccgcctgcaagtcctaagacgccaatcgaaaagaaacacgcggatgaaatcgataagtatatacaaggattggattacaataaaaacaatgtattagtataccacggagatgcagtgacaaatgtgccgccaagaaaaggttataaagatggaaatgaatatatcgttgtggagaaaaagaagaaatccatcaatcaaaataatgcagatatccaagttgtgaatgcaatttcgagcctaacatatccaggtgctctcgtgaaagcgaattcggaattagtagaaaatcaacccgatgttcttcctgtcaaacgtgattcattaacacttagcattgatttgccaggaatgactaatcaagacaataaaattgttgtaaaaaatgctactaaatcgaacgttaacaacgcagtaaatacattagtggaaagatggaatgaaaaatatgctcaagcttatccaaatgtaagtgcaaaaattgattatgatgacgaaatggcttacagtgaatcacaattaattgcaaaatttggtacggcatttaaagctgtaaataatagcttgaatgtaaacttcggcgcaatcagtgaagggaaaatgcaagaagaagtcattagttttaaacaaatttactataacgtgaatgttaatgaacctacaagaccttccagatttttcggcaaagctgttactaaagagcagttgcaagcgcttggagtgaatgcagaaaatcctcctgcatatatctcaagtgtggcatatggccgtcaagtttatttgaaattatcaactaattcccatagtactaaagtaaaagctgcttttgacgctgccgtaagtgggaaatctgtctcaggtgatgtagaactgacaaatatcatcaaaaattcttccttcaaagccgtaatttacggtggctccgcaaaagatgaagttcaaatcatcgacggtaacctcggagacttacgagatattttgaaaaaaggtgctacttttaaccgggaaacaccaggagttcccattgcctatacaacaaacttcttaaaagacaatgaattagctgttattaaaaacaactcagaatatattgaaacaacttcaaaagcttatacagatggaaaaatcaacatcgatcactctggaggatacgttgctcaattcaacatctcttgggatgaaataaattatgatcctgaaggtaacgaaattgttcaacataaaaactggagcgaaaacaataaaagtaagctagctcatttcacatcgtccatctatttgccaggtaacgcaagaaatattaatgtttacgctaaagaatgcactggtttagcttgggaatggtggagaacggtaattgatgaccggaacctaccgcttgtgaaaaatagaaatatctccatctggggcactacactttatccgaaatatagtaatagtgtagataatccaatcgaataa

SEQ ID NO: 33 - DNA, 1593 bp, Listeria seeligeri
atgaaaatatttggtttagttatcatgtcgttgctatttgttagtttgccaataacacaacaacctgaagcgagggatgtccccgcgtacgatagaagcgaggtgactatatctcctgctgaaacaccagagtccccaccggcaacaccaaaaacacctgtagagaaaaagcatgcggaagaaattaataaatatatttggggattaaactatgataaaaatagtattctggtctatcaaggtgaagcagttacaaacgttccaccgaaaaagggctacaaagatggcagtgaatatattgtcgttgaaaaaaagaaaaaaggtatcaatcaaaacaatgcagacatttctgtcataaatgcaatttcgagccttacttatcctggagcgttggtaaaagcaaatagagaattagtagaaaatcaacctaatgtactaccagtaaaacgagattcacttacattaagtgtagatttaccaggaatgactaaaaaagataataaaatattcgttaaaaaccctacaaagtcaaacgtaaataatgccgtgaatacattagtagagcgttggaatgataagtattcaaaagcgtatcctaatattaatgcaaaaattgattattccgatgaaatggcttatagtgaatcacaattaattgccaaatttgggactgcctttaaagctgttaataatagtttgaatgtaaattttgaggcaattagtgatgggaaagtacaagaagaagtcattagttttaagcaaatttattataatattaacgttaatgaacctacaagtccttccaaattctttgggggtagtgttaccaaagaacaactagatgctttaggtgtaaatgccgaaaatcctcctgcttacatttctagtgttgcttacggtcgccaagtttatgtgaaactatcctctagctcgcatagtaacaaagttaaaactgctttcgaggcggcgatgagtggcaaatcagtgaaaggggatgtagaattaacaaatattataaaaaattcttcttttaaagcagtcatttatggtggctcagcgaaagaagaggttgaaattattgatggcaatttaggcgaacttcgagatattttgaaaaaagggtccacttatgatagagaaaaccctggcgttccgatctcgtacacaactaactttttgaaagataatgacttagcggttgttaaaaacaactcagaatatatcgaaacaacttcgaaatcttatacagatggaaaaattaatattgatcattctggtggttatgtagcccaattcaatatatcttgggatgaagtaagttatgacgagaacggaaatgaaataaaagttcataagaaatggggcgaaaattataagagtaagttagctcatttcacttcttctatctatttgccaggaaatgcgagaaatattaacatctatgcaagagaatgtaccggcttgttttgggaatggtggagaactgttatagatgacagaaacttaccattagtaaaaaatagaaatgtatctatttggggtacaacgctttacccaagacattctaataatgtagataatccgattcagtag

SEQ ID NO: 34 - DNA, 1494 bp, Streptococcus suis
atgagaaaaagttcgcacttgattttaagctcaatagtcagtttggcactcgtaggggtcacaccattgagtgttcttgcagattccaaacaagatattaatcagtattttcaaagcttgacttacgagccacaagagattcttacaaatgagggagaatacattgataatccgccagcaacaactggtatgttagaaaacggacgttttgtagtacttcgcagagaaaagaagaatattacgaacaatagtgcagatattgctgttattgatgctaaggctgcaaatatttatccaggtgctttattgcgtgctgaccaaaatcttctggataataatccaacgcttatcagtattgcgcggggagatctgacgcttagtttgaatttacctggtttggccaatggggatagccacactgttgtaaattctccaacaagaagtactgttcgaacaggggtgaataaccttctgtctaaatggaataatacgtatgctggagagtatggcaatacccaagcagagcttcaatatgatgaaacaatggcatacagtatgtcacaattgaaaacgaagttcggaacctcttttgaaaaaattgctgtaccattagatatcaattttgatgccgtgaattcgggtgaaaaacaggttcagattgttaactttaaacaaatttattatacagttagtgttgatgaaccagaatctccaagcaagctttttgcagaagggacaactgtagaagatttgaaacgaaatgggataacagatgaggtacctcctgtttatgtttccagcgtttcttatggacgctctatgttcatcaagttagaaactagcagtaggagtacccaagttcaagccgcatttaaagcagccatcaaaggcgttgatattagtggcaatgctgagtatcaagacattctgaaaaatacttcattctctgcttatatttttggtggggatgcaggtagcgcggctactgttgtgagcggaaatattgaaacactgaagaagattattgaagaaggtgcaagatacggaaaactcaatccaggtgttccgatttcgtattcaaccaactttgtcaaagacaatagacctgctcagattttgagcaattcagagtacatagaaacaacttcaacagtccataatagcagtgcattgacattggatcattcaggtgcttatgttgcgaaatacaacattacttgggaagaagtatcttacaatgaagctggagaagaagtttgggaaccaaaagcttgggataagaatggtgtaaatctgacctcacactggagtgaaaccattcaaattccaggaaatgctcgcaatcttcatgtcaatattcaagaatgtacaggattagcatgggagtggtggagaacagtttatgacaaagatttaccacttgttggtcaacgtaaaataaccatctggggaacaacgttatacccacagtatgcggatgaggtgatagagtaa

SEQ ID NO: 35 - DNA, 1398 bp, Streptococcus mitis
atggcaaataaagcagtaaatgactttatactagctatggattacgataaaaagaaactcttgacccatcagggagaaagtattgaaaatcgtttcatcaaagaggggaatcagctacccgatgagtttgttgttatcgaaagaaagaagcggagcctgtcgacaaatacaagtgatatttctgtgacagctaccaacgacagtcgcctctatcctggagcacttctcgtagtggatgagaccttgttagagaataatcccactcttcttgcggtcgatcgtgctccgatgacttatagtattgatttgcctggtttggcaagtagtgatagctttctccaagtagaagatcccagcaattcaagtgttcgcggagcggtaaacgatttgttggctaagtggcatcaagattatggtcaggtcaataatgtcccagctagaatgcagtatgaaaaaatcacggctcacagcatggaacaactcaaggtcaagtttggttctgactttgaaaagacagggaattctcttgatattgattttaactctgtccattcgggcgaaaagcagattcagattgttaattttaagcagatttattatacagtcagcgtagatgctgttaaaaatccaggagatgtatttcaagatactgtaacggtagaggatttgaggcagagaggaatttctgccgatcgtcctttggtctatatttcgagtgttgcttatgggcgccaggtttatctcaagttggagaccacgagtaagagtgatgaagtcgaggctgcttttgaagctttgataaaaggagtcaaggtagctcctcagacagagtggaagcagattttggacaatacagaagtgaaggcggttattttagggggcgacccgagttcgggtgcccgagttgtaacaggcaaggtggatatggtagaggacttgattcaagaaggcagtcgctttacagccgatcatccaggtttgccgatttcttatacaacttcttttttacgggacaatgtagttgcgacctttcaaaacagtacagactatgttgagactaaggtgacagcctacagaaacggagatttactgctggatcatagtggtgcctatgttgctcaatattacattacttgggatgaattatcctatgattatcaaggtaaggaagttttgactcctaaggcttggaacagaaatgggcaggatttgacggctcattttaccactagtattcctttaaaagggaatgttcgcaatctctctgtcaaaattagagagtgtaccggacttgcctgggaatggtggcgtacggtttatgaaaaaaacgatttgcccctagtgcgtaagcggacgatttctatttggggaacgactctttatcctcaggtagaggat

SEQ ID NO: 36 - DNA, 1599 bp, Streptococcus intermedius
atgaaaactaagcagaatattgctcgcaaattgtcaagagttgttttattaagcactctcgttctctcttcggcagcaccgatttcagctgcattcgctgaaacacctaccaaaccaaaagcagctcaaacagagaaaaaacccgaaaagaaaccggaaaacagcaactctgaagctgcaaaaaaagctctgaatgattatatttggggattgcagtatgataaactaaacattttaacacaccaaggtgaaaaattgaaaaaccactctagccgcgaggcatttcatcgcccaggtgagtatgttgttatcgaaaagaaaaaacaaagcatttcaaacgcaacatctaagttatctgtaagttcagcaaatgatgaccgcatcttcccaggtgcattgctaaaagcggaccaaagtttgttagaaaatcttccaaccctaatcccagttaatcgcggcaaaacaactattagtgtaaacttaccgggattgaaaaatggcgaaagtaatcttacagttgaaaatccatccaacagtacagttcgaacagctgttaacaatttagttgaaaaatggattcaaaaatactctaaaactcatgctgtgccagctagaatgcaatatgaatctattagcgcccaaagcatgagccaattacaagcaaaatttggtgctgatttctcaaaagtcggtgcaccacttaatgttgacttctcatctgttcacaaaggtgaaaaacaagtatttattgcgaactttagacaagtttactacacagctagcgtagactctccaaatagtccttctgcactctttggctctggtatcacaccaactgatttaatcaatcgtggagttaattctaaaaccccaccagtttatgtttcaaatgtatcatatggccgtgcaatgtatgtgaaatttgaaactacaagcaagagtacaaaagtacaagccgctattgatgctgttgttaaaggagcaaaacttaaagctggaacagaatatgaaaatattctaaaaaatactaaaatcactgctgttgttctcggtggtaacccaggtgaagcttctaaagtcatcacaggtaatattgatactttgaaagatttgatccaaaaaggtagcaatttcagtgctcaaagtccagctgtaccaatctcttacactacttcttttgtaaaagacaattctattgcaactatccaaaacaacacagactacatcgaaacaaaagtaacatcctataaagatggtgctctcaccctcaatcatgatggtgctttcgttgcacgcttctatgtttattgggaagaactcggacatgatgctgatggctacgaaactattcgctcaagatcttggagtggaaatggctacaatcgcggtgcacactattctacaactctccgtttcaagggaaatgttagaaacattcgcgtaaaagtactaggagccactggactagcttgggagccttggagactgatctatagcaagaacgatcttcctttggttccacaaagaaacattagcacttggggaacaacccttcatccacagtttgaagataaagttgtgaaagataacactgattaa

SEQ ID NO: 37 - DNA, 1998 bp, Streptococcus mitis
atgaatcaagaaaaacgtttgcatcgctttgtcaaaaagtgtggactcggtgtgtgtagtgctgttgttgcggcctttttattgaacgctcagggagtagctttggctacagagcaagggaatcgtccagttgagaccgaaaacatcgctcgtggaaaacaagctagtcaaagttctactgcttatggaggagctgctgcacgagcagtggacggtaatgttgacagtgactatgggcaccattctgtaacgcacacaaactttgaagacaatgcttggtggcaagttgatcttggaaaaacagagaatgttggaaaagttaaactctacaatcgtggagatgggaatgtagctaatcgtctttccaattttgatgttgttttgttaaatgaagcaaaacaagaagttgctcgtcaacactttgatagtttgaatgggaaggcagaacttgaagttttcttcaccgccaaagccgctcgttatgtaaaagtggagttgaaaactaaaaataccccattgagcttggcagaagtggaagtattccgttcagcaacaactcaagttggacaggatagaactgcaccagtagtagatcaaacatcagcattgaaagactacctttttggcttagcttataatcctttggatattttaactcgcaagggagaaaccttagaaaatcgctacaacacaagtgctaaggaacaaaatggagagtttgtcgttgtagaaaaaatcaagaaaaccctctctacaggcacagcagatgtttccatcaatggaaatcaaaatgtcttcctaggtggcttgtataaggcaaaccaaaatctgctagaaaatcagccagaattgattagtcttgcccgtgcaaaggggacagtcagcgtcgatttacctggtatgattcagtctgacagccgaattgaagcagatcctacaactagtggtatgcagtctgcgatgaataccttggttgaaagatggacaaagaattactcatctagccattccgttcctgcccgtgttcagtatgaatcaactacagcctatagcatgaatcaattgaaagcaaaatttggtgcagactttgaaaaagcaggtgcaccgctcaagattgactttgaggctgtgcaaaagggtgaaaagcaaattgaagttgtaaactttaaacaaatctactatacagcgacatttgatgcaccgaccaatccagcggctgtatttgacaagagtgtgacacctgaagatttaaaacaaagaggcgttgattcacaaactccacctgtatatgtatcaaatgtttcttacggacgtcaaatctatgttaagtttgagtcagcaagtaagtctactgaattaaaagcagctattaatgcggttatcaaaggcgcaacaattgctccaaattctgaatggagccgtctattgaagaatacttctgtaacagcggtaattgtaggaggtaatgctagcggtgccgccaaagttgtcacaggaacagtcgaaaacttgaaggaactcatcagagaaggagctaactttagcgctcaaagtccagctgtgccaatctcatataagactgccttcctaaaagataatgcccaagcaactttacaaaatagtacagactatatcgaaacgaaggttacttcttacaaaaatggtttcttgaaacttcatcataagggtgcttatgttgcgcgttactacatctattgggatgaaattacatatgatgaacaaggaaatccagaaatccgttcacgtcaatgggaagataacggaaaaaacagaacttcaggcttccaaacagagattcaatttagaggaaatgtccgtaatcttcgcatcaaggttcaagaaaagacgggtcttgtatgggaaccatggcgtacagtttacaaccgcacagacttaccactagtacaacagcgtacaattacacattggggaacaactctaaaccctaaagttgatgaaaaaattgtgaatgagtaa

SEQ ID NO: 38 - DNA, 1605 bp, Arcanobacterium pyogenes
atgaaacgaaaggcttttgcatcgctagtggcgagtgtagtcgcagcagcaactgtcacgatgcccacagcatcttttgctgccggattgggaaacagctcgggattgacggacggcttgtcagcgccgcgagcctccatctccccgacggataaagttgaccttaagtcggcgcaagagaccgacgagacgggcgtcgataagtacattcgtggtctgaaatacgatccctctggtgtacttgcagtcaagggtgagtctattgaaaatgtgccggttaccaaggatcagctcaaggacggcacctacacggtatttaagcatgaacgcaagagttttaacaatttgcgttcggacatctctgcgttcgatgcgaacaacgcccacgtctatcctggcgcgctcgtgttagcaaataaagatcttgcaaaaggtagtccgacttcgatcggaattgcacgtgctccgcaaactgtcagcgtcgacttgccaggattagttgacggtaagaataaggtcgtcatcaacaatcccacgaagagttccgtgactcaaggactgaacggccttctcgacggttggattcagcgcaatagcaagtatcctgaccatgctgcaaagatctcctacgatgagactatggtgacgtcaaagcgtcaactggaggcaaagcttggcctcggatttgaaaaggtctcagccaagctcaacgtggacttcgatgcaattcataagcgtgaacggcaggtggctatcgcttccttcaaacagatttactacacggctagcgtagatacaccgacatctccacatagcgttttcggcccgaatgtcaccgcacaggatttgaaagatcggggagtcaataacaagaatcctctaggatacatttcgtcggtcagctatggacgccagatttttgtcaagctggaaacgacctcgacttccaatgatgtacaagcggcttttagcggcctgttcaaagctaagttcggcaatctttccacagagttcaaggctaagtatgccgatatcctgaacaagacccgagctactgtgtacgctgttggtggcagcgctagaggcggagttgaagttgcaactggcaatatcgatgcactcaagaagatcatcaaggaggaaagcacctactctacgaaggttcctgccgtgcccgtttcctatgccgtcaatttcttgaaggataatcagttggcagctgttaggagcagcggtgattacattgaaaccactgcaacgacttacaagtctggtgagatcaccttccgccatggcggtggctacgtcgcaaagttcaggctgaagtgggacgagatcagctacgacccgcagggcaaggaaatccgtacacccaagacgtggagcgggaattgggcagcccgcacccttggcttccgtgagactattcaacttccagcaaacgcgcgcaacatccatgtggaagcaggcgaggcaactggcctagcgtgggatccgtggtggaccgttatcaataagaagaatctccccttggtgccacatcgagagatcgtccttaagggcacgacgctcaatccctgggtcgaggacaatgtcaaatcctag

SEQ ID NO: 39 - protein, 11 aa, Streptococcus pneumoniae
ECTGLAWEWWR

SEQ ID NO: 40 - protein, 471 aa, Streptococcus pneumoniae
MANKAVNDFILAMNYDKKKLLTHQGESIENRFIKEGNQLPDEFVVIERKKRSLSTNTSDISVTATNDSRLYPGALLVVDETLLENNPTLLAVDRAPMTYSIDLPGLASSDSFLQVEDPSNSSVRGAVNDLLAKWHQDYGQVNNVPARMQYEKITAHSMEQLKVKFGSDFEKTGNSLDIDFNSVHSGEKQIQIVNFKQIYYTVSVDAVKNPGDVFQDTVTVEDLKQRGISAERPLVYISSVAYGRQVYLKLETTSKSDEVEAAFEALIKGVKVAPQTEWKQILDNTEVKAVILSGDPSSGARVVTGKVDMVEDLIQEGSRFTADHPGLPISYTTSFLRDNVVATFQNSTDYVETKVTAYRNGDLLLDHSGAYVAQYYITWDELSYDHQGKEVLTPKAWDRNGQDLTAHFTTSIPLKGNVRNLSVKIRECTGLAWEWWRTVYEKTDLPLVRKRTISIWGTTDYPQVEDKVEND